European Patent Application EP 4 134 093 A1, published February 15, 2023. Title: A Peptide for preventing or treating hair loss and the uses thereof. Applicant: Daegu Gyeongbuk Institute of Science and Technology. The sequence listing filed with the application follows.

SEQUENCE LISTING (4 sequences)

SEQ ID NO: 1 - protein, 19 aa, Artificial Sequence
  MLP amino acid peptide
LHVDKAVSGLRSLTTLLRA

SEQ ID NO: 2 - protein, 19 aa, Artificial Sequence
  MLP-C amino acid peptide
RHVKKRVKGLKSLTTLLRA

SEQ ID NO: 3 - protein, 19 aa, Artificial Sequence
  MLP-H amino acid peptide
LHVLKAVSGLLTLTMIRRA

SEQ ID NO: 4 - protein, 19 aa, Artificial Sequence
  Scr amino acid peptide(negative control)
MELSGRTLGLILKLRQSAT